European Patent Specification EP 4 189 393 B1, published April 15, 2026. Title: RELIABLE AND SCALABLE METHODS OF DETECTION AND PLATFORM FOR CONSUMER MEDICAL DEVICES. Applicant: Simple Healthkit, Inc. The sequence listing filed with the application follows.

SEQUENCE LISTING (90 sequences)

SEQ ID NO: 1 - protein, 243 aa, Chlamydia trachomatis (strain D/UW-3/Cx)
MKNILSWMLMFAVALPIVGCDNGGGSQTSATEKSMVEDSALTDNQKLSRTFGHLLSRQLSRTEDFSLDLVEVIKGMQSEIDGQSAPLTDTEYEKQMAEVQKASFEAKCSENLASAEKFLKENKEKAGVIELEPNKLQYRVVKEGTGRVLSGKPTALLHYTGSFIDGKVFDSSEKNKEPILLPLTKVIPGFSQGMQGMKEGEVRVLYIHPDLAYGTAGQLPPNSLLIFEVKLIEANDDNVSVTE

SEQ ID NO: 2 - protein, 264 aa, Chlamydia trachomatis
MGNSGFYLYNTENCVFADNIKVGQMTEPLKDQQIILGTKSTPVAAKMTASDGISLTVSNNSSTNASITIGLDAEKAYQLILEKLGNQILDGIADTIVDSTVQDILDKITTDPSLGLLKAFNNFPITNKIQCNGLFTPSNIETLLGGTEIGKFTVTPKSSGSMFLVSADIIASRMEGGVVLALVREGDSKPCAISYGYSSGVPNLCSLRTSITNTGLTPTTYSLRVGGLESGVVWVNALSNGNDILGITNTSNVSFLEVIPQTNA

SEQ ID NO: 3 - protein, 88 aa, Chlamydia trachomatis
MKKTALLAALCSVVSLSSCCRIVDCCFEDPCAPIQCSPCESKKKDVDGGCNSCNGYVPACKPCGGDTHQDAEHGPQAREIPVDGKCRQ

SEQ ID NO: 4 - protein, 512 aa, Chlamydia trachomatis (strain D/UW-3/Cx)
MPHDNNEMHRNTIHQLFTGLDKAYQIVKGFYGPAYSSSSKDFFKGRGYHILSRIELSDPFERIGVYFARSLAKRIHKRHADGVISSVILLRAFLKASIPFIDQGLSPRLLASALASQKEAVCAYLHSHSFLLKDASKVLGLIRSHLPDPLIGEAFAEAVAYTGHEGAVALSQRSGSTLHLVKGIQTQKGYRVPSFFPHDSFHENPIVAPKIFVTDQKIHCLFPFLPLLKKFSEEQTPLIIFCKEIAPDPLATCIANRIAGLLDVLVVTIPDTTLLEDIALLTGTTVFSSPPFSNKPPIELPLLGSCTWAELSRDHTLLVCENLVPEVVKLKVRQLDHAIHNAEDETSRKLLKKRKHRLENSIAIIPVKQDTTPLHELALKTLNSTQESGFVLGGGAALLYATQSLSSSPEHSQEEQAAVQILQTACRTLLEQLVNSVYMDGKLVADKLCSLGTPSLGFNVVSQQIEDMISAGIITPLNVVLDIFSCSLHTAVDLLLASFTTPPTPAAKEKKT

SEQ ID NO: 5 - protein, 394 aa, Chlamydia trachomatis serovar L2 (strain 434/Bu/ATCC VR-902-B)
MKKLLKSVLVFAALSSASSLQALPVGNPAEPSLMIDGILWEGFGGDPCDPCTTWCDAISMRMGYYGDFVFDRVLQTDVNKEFQMGAKPTTATGNAAAPSTCTARENPAYGRHMQDAEMFTNAAYMALNIWDRFDVFCTLGATSGYLKGNSASFNLVGLFGDNENHATVSDSKLVPNMSLDQSVVELYTDTTFAWSAGARAALWECGCATLGASFQYAQSKPKVEELNVLCNAAEFTINKPKGYVGQEFPLDLKAGTDGVTGTKDASIDYHEWQASLALSYRLNMFTPYIGVKWSRASFDADTIRIAQPKSATTVFDVTTLNPTIAGAGDVKASAEGQLGDTMQIVSLQLNKMKSRKSCGIAVGTTIVDADKYAVTVETRLIDERAAHVNAQFRF

SEQ ID NO: 6 - protein, 102 aa, Chlamydia trachomatis (strain D/UW-3/Cx)
MSDQATTLKIKPLGDRILVKREEEASTARGGIILPDTAKKKQDRAEVLALGTGKKDDKGQQLPFEVQVGNIVLIDKYSGQELTVEGEEYVIVQMSEVIAVLQ

SEQ ID NO: 7 - protein, 102 aa, Chlamydia trachomatis; identical to SEQ ID NO: 6

SEQ ID NO: 8 - protein, 89 aa, Chlamydia trachomatis
MLKPLKDRVVIQMVEQEEKTAGGLFLPTAAQEKLQFATVLAVSEFTEEKDRQVQVGDRVVFEKYTGTEVKLDGQEYIIVKEQDIIAIVQ

SEQ ID NO: 9 - DNA, 58 bp, DNA-based aptamer
atttcacaatatttagtcagccatgaccggtgcagtttatgagtattgtgttcagaga

SEQ ID NO: 10 - DNA, 58 bp, DNA-based aptamer
attcactcgtcgggaaactatgggcgtacggtgctcggtttccttctctctgagtaga

SEQ ID NO: 11 - DNA, 58 bp, DNA-based aptamer
attgggggcgggagggggatggcggaggtttgttgtctgttcggggagctgtgtaaga

SEQ ID NO: 12 - DNA, 56 bp, DNA-based aptamer
agggggcaggggggttgactttaccttatgcttaaagggggtgggctcgggaagat

SEQ ID NO: 13 - DNA, 55 bp, DNA-based aptamer
agggggagaacgggggggcttgggttggggatggatgtgggaggccggtcgagat

SEQ ID NO: 14 - DNA, 58 bp, DNA-based aptamer
tggcgcggacgtactggcgaattggtgagcctcgggctgggtggggggttagggagat

SEQ ID NO: 15 - DNA, 55 bp, DNA-based aptamer
ctcacactattttttggcataggtgtcgagggtggacggggcggggcggtgagat

SEQ ID NO: 16 - DNA, 56 bp, DNA-based aptamer
gagttaagtttgagtgttgtcgagggtggacggggtggggcaagctagtgtgagat

SEQ ID NO: 17 - protein, 243 aa, Chlamydia trachomatis (strain D/UW-3/Cx); identical to SEQ ID NO: 1

SEQ ID NO: 18 - protein, 264 aa, Chlamydia trachomatis; identical to SEQ ID NO: 2

SEQ ID NO: 19 - protein, 660 aa, Chlamydia trachomatis serovar L2 (strain 434/Bu/ATCC VR-902-B)
MSEKRKSNKIIGIDLGTTNSCVSVMEGGQPKVIASSEGTRTTPSIVAFKGGETLVGIPAKRQAVTNPEKTLASTKRFIGRKFSEVESEIKTVPYKVAPNSKGDAVFDVEQKLYTPEEIGAQILMKMKETAEAYLGETVTEAVITVPAYFNDSQRASTKDAGRIAGLDVKRIIPEPTAAALAYGIDKEGDKKIAVFDLGGGTFDISILEIGDGVFEVLSTNGDTHLGGDDFDGVIINWMLDEFKKQEGIDLSKDNMALQRLKDAAEKAKIELSGVSSTEINQPFITIDANGPKHLALTLTRAQFEHLASSLIERTKQPCAQALKDAKLSASDIDDVLLVGGMSRMPAVQAVVKEIFGKEPNKGVNPDEVVAIGAAIQGGVLGGEVKDVLLLDVIPLSLGIETLGGVMTPLVERNTTIPTQKKQIFSTAADNQPAVTIVVLQGERPMAKDNKEIGRFDLTDIPPAPRGHPQIEVTFDIDANGILHVSAKDAASGREQKIRIEASSGLKEDEIQQMIRDAELHKEEDKQRKEASDVKNEADGMIFRAEKAVKDYHDKIPAELVKEIEEHIEKVRQAIKEDASTTAIKAASDELSTRMQKIGEAMQAQSASAAASSAANAQGGPNINSEDLKKHSFSTRPPAGGSASSTDNIEDADVEIVDKPE

SEQ ID NO: 20 - protein, 232 aa, Chlamydia trachomatis serovar L2 (strain 434/Bu/ATCC VR-902-B)
MTKHGKRIRGIQETYDLAKSYSLGEAIDILKQCPTVRFDQTVDVSVKLGIDPRKSDQQIRGSVSLPHGTGKVLRILVFAAGDKAAEAIEAGADFVGSDDLVEKIKGGWVDFDVAVATPDMMREVGKLGKVLGPRNLMPTPKAGTVTTDVVKTIAELRKGKIEFKADRAGVCNVGVAKLSFDSAQIKENVEALCAALVKAKPATAKGQYLVNFTISSTMGPGVTVDTRELIAL

SEQ ID NO: 21 - protein, 1014 aa, Chlamydia trachomatis serovar A (strain A2497)
MMQTSFHKFFLSMILAYSCCSLNGGGYAAEIMVPQGIYDGETLTVSFPYTVIGDPSGTTVFSAGELTLKNLDNSIAALPLSCFGNLLGSFTVLGRGHSLTFENIRTSTNGAALSDSANSGLFTIEGFKELSFSNCNSLLAVLPAATTNNGSQTPTTTSTPSNGTIYSKTDLLLLNNEKFSFYSNLVSGDGGAIDAKSLTVQGISKLCVFQENTAQADGGACQVVTSFSAMANEAPIAFVANVAGVRGGGIAAVQDGQQGVSSSTSTEDPVVSFSRNTAVEFDGNVARVGGGIYSYGNVAFLNNGKTLFLNNVASPVYIAAEQPTNGQASNTSDNYGDGGAIFCKNGAQAAGSNNSGSVSFDGEGVVFFSSNVAAGKGGAIYAKKLSVANCGPVQFLGNIANDGGAIYLGESGELSLSADYGDMIFDGNLKRTAKENAADVNGVTVSSQAISMGSGGKITTLRAKAGHQILFNDPIEMANGNNQPAQSSEPLKINDGEGYTGDIVFANGNSTLYQNVTIEQGRIVLREKAKLSVNSLSQTGGSLYMEAGSTLDFVTPQPPQQPPAANQLITLSNLHLSLSSLLANNAVTNPPTNPPAQDSHPAVIGSTTAGSVTISGPIFFEDLDDTAYDRYDWLGSNQKIDVLKLQLGTQPPANAPSDLTLGNEMPKYGYQGSWKLAWDPNTANNGPYTLKATWTKTGYNPGPERVASLVPNSLWGSILDIRSAHSAIQASVDGRSYCRGLWVSGVSNFFYHDRDALGQGYRYISGGYSLGANSYFGSSMFGLAFTEVFGRSKDYVVCRSNHHACIGSVYLSTKQALCGSYVFGDAFIRASYGFGNQHMKTSYTFAEESDVRWDNNCLVGEIGVGLPIVITPSKLYLNELRPFVQAEFSYADHESFTEEGDQARAFRSGHLMNLSVPVGVKFDRCSSTHPNKYSFMGAYICDAYRTISGTQTTLLSHQETWTTDAFHLARHGVIVRGSMYASLTSNIEVYGHGRYEYRDTSRGYGLSAGSKVRF

SEQ ID NO: 22 - protein, 547 aa, Chlamydia trachomatis
MNKLIRRAVTIFAVTSVASLFASGVLETSMAESLSTNVISLADTKAKDNTSHKSKKARKNHSKETLVDRKEVAPVHESKATGPKQDSCFGRMYTVKVNDDRNVEITQAVPEYATVGSPYPIEITATGKRDCVDVIITQQLPCEAEFVRSDPATTPTADGKLVWKIDRLGQGEKSKITVWVKPLKEGCCFTAATVCACPEIRSVTKCGQPAICVKQEGPENACLRCPVVYKINVVNQGTAIARNVVVENPVPDGYAHSSGQRVLTFTLGDMQPGEHRTITVEFCPLKRGRATNIATVSYCGGHKNTASVTTVINEPCVQVSIAGADWSYVCKPVEYVISVSNPGDLVLRDVVVEDTLSPGVTVLEAAGAQISCNKVVWTVKELNPGESLQYKVLVRAQTPGQFTNNVVVKSCSDCGTCTSCAEATTYWKGVAATHMCVVDTCDPVCVGENTVYRICVTNRGSAEDTNVSLMLKFSKELQPVSFSGPTKGTITGNTVVFDSLPRLGSKETVEFSVTLKAVSAGDARGEAILSSDTLTVPVSDTENTHIY

SEQ ID NO: 23 - protein, 792 aa, Neisseria gonorrhoeae
MKLKQIASALMMLGISPLAFADFTIQDIRVEGLQRTEPSTVFNYLPVKVGDTYNDTHGSAIIKSLYATGFFDDVRVETADGLLLLTVIVCPTIGSLNITGAKMLQNDAIKKNLESFGLAQSQYFNQATLNQAVAGLKEEYLGRGKLNIQITPKVTKLARNRVDIDITIDEGKSAKITDIEFEGNQVYSDRKLMRQMSLTEGGIWTWLTRSDRFDRQKFAQDMEKVTDFYQNNGYFDFRILDTDIQTNEDKTRQTIKITVHEGGRFRWGKVSIEGDTNEVPKAELEKLLTMKPGKWYERQQMTAVLGEIQNRMGSAGYAYSEISVQPLPNAGTKTVDFVLHIEPGRKIYVNEIHITGNNKTRDEVVRRELRQMESAPYDTSKLQRSKERVELLGYFDNVQFDAVPLAGTPDKVDLNMSLTERSTGSLDLSAGWVQDTGLVMSAGVSQDNLFGTGKSAALRASRSKTTLNGSLSFTDPYFTADGVSLGYDIYGKAFDPRKASTSVKQYKTTTAGGGVRMGIPVTEYDRVNFGLAAEHLTVNTYNKAPKRYADFIKQYGKTDGADGSFKGLLYKGTVGWGRNKTDSALWPTRGYLTGVNAEIALPGSKLQYYSATHNQTWFFPLSKTFTLMLGGEVGIAGGYGRTKEIPFFENFYGGGLGSVRGYESGTLGPKVYDEYGEKISYGGNKKANVSAELLFPMPGAKDARTVRLSLFADAGSVWDGRTYTAAENGNNKSVYSENAHKSTFTNELRYSAGGAVTWLSPLGPMKFIYAYPLKKKPEDEIQRFQFQLGTTF

SEQ ID NO: 24 - protein, 792 aa, Neisseria gonorrhoeae
MKLKQIASALMMLGISPLAFADFTIQDIRVEGLQRTEPSTVFNYLPVKVGDTYNDTHGSAIIKSLYATGFFDDVRVETADGQLLLTVIERPTIGSLNITGAKMLQNDAIKKNLESFGLAQSQYFNQATLNQAVAGLKEEYLGRGKLNIQITPKVTKLARNRVDIDITIDEGKSAKITDIEFEGNQVYSDRKLMRQMSLTEGGIWTWLTRSDRFDRQKFAQDMEKVTDFYQNNGYFDFRILDTDIQTNEDKTRQTIKITVHEGGRFRWGKVSIEGDTNEVPKAELEKLLTMKPGKWYERQQMTAVLGEIQNRMGSAGYAYSEISVQPLPNAGTKTVDFVLHIEPGRKIYVNEIHITGNNKTRDEVVRRELRQMESAPYDTSKLQRSKERVELLGYFDNVQFDAVPLAGTPDKVDLNMSLTERSTGSLDLSAGWVQDTGLVMSAGVSQDNLFGTGKSAALRASRSKTTLNGSLSFTDPYFTADGVSLGYDIYGKAFDPRKASTSVKQYKTTTAGGGVRMGIPVTEYDRVNFGLAAEHLTVNTYNKAPKRYADFIKQYGKTDGADGSFKGLLYKGTVGWGRNKTDSALWPTRGYLTGVNAEIALPGSKLQYYSATHNQTWFFPLSKTFTLMLGGEVGIAGGYGRTKEIPFFENFYGGGLGSVRGYESGTLGPKVYDEYGEKISYGGNKKANVSAELLFPMPGAKDARTVRLSLFADAGSVWDGRTYTAAENGNNKSVYSENAHKSTFTNELRYSAGGAVTWLSPLGPMKFSYAYPLKKKPEDEIQRFQFQLGTTF

SEQ ID NO: 25 - protein, 326 aa, Neisseria gonorrhoeae
MKKSLIALTLAALPVAAMADVTLYGTIKAGVETSRSVAHHGAQADRVKTATEIADLGSKIGFKGQEDLGNGLKAIWQLEQKAYVSGTDTGWGNRQSFIGLKGGFGKVRVGRLNSVLKDTGGFNPWEGKSYYLGLSNIAQPEERHVSVRYDSPEFAGFRAVQYVPNDNSGKNHSESYHAGFNYKNSGFFVQYAGFYKRHSYTTEKHQVHRLVGGYDHDALYASVAVQQQDAKLTWRNDNSHNSQTEVAATAAYRFGNVTPRVSYAHGFKGSVYDADNDNTYDQVVVGAEYDFSKRTSALVSAGWLQRGKGTEKFVATVGGVGLRHKF

SEQ ID NO: 26 - protein, 392 aa, Neisseria gonorrhoeae
MKRQALAAMIASLFALAACGGEQAAQAPAETPAASAEAASSAAQATAETPAGELPVIDAVTTHAPEVPPAIDRDYPAKVRVKMETVEKTMKMDDGVEYRYWTFDGDVPGRMIRVREGDTVEVEFSNNPSSTVPHNVDFHAATGQGGGAAATFTAPGRTSTFSFKALQPGLYIYHCAVAPVGMHIANGMYGLILVEPKEGLPKVDKEFYIVQGDFYTKGKKGAQGLQPFDMDKAVAEQPEYVVFNGHVGSIAGDNALKAKAGETVRMYVGNGGPNLVSSFHVIGEIFDKVYVEGGKLINENVQSTIVPAGGSAIVEFKVDIPGSYTLVDHSIFRAFNKGALGQLKVEGAENPEIMTQKLSDTAYAGSGAASAPAASAPAASAPAASASEKSVY

SEQ ID NO: 27 - protein, 467 aa, Neisseria gonorrhoeae
MNTTLKTTLTSVAAAFALSACTMIPQYEQPKVEVAETFQNDTSVSSIRAVDLGWHDYFADPRLQKLIDIALERNTSLRTAVLNSEIYRKQYMIERNNLLPTLAANANGSRQGSLSGGNVSSSYNVGLGAASYELDLFGRVRSSSEAALQGYFASVANRDAAHLSLIATVAKAYFNERYAEEAMSLAQRVLKTREETYNAVRIAVQGRRDFRRRPAPAEALIESAKADYAHAARSREQARNALATLINRPIPEDLPAGLPLDKQFFVEKLPAGLSSEVLLDRPDIRAAEHALKQANANIGAARAAFFPSIRLTGSVGTGSVELGGLFKSGTGVWAFAPSITLPIFTWGTNKANLDVAKLRQQAQIVAYESAVQSAFQDVANALAAREQLDKAYDALSKQSRASKEALRLVGLRYKHGVSGALDLLDAERSSYSAEGAALSAQLTRAENLADLYKALGGGLKRDTQTGK

SEQ ID NO: 28 - protein, 594 aa, Neisseria gonorrhoeae (strain ATCC 700825 / FA 1090)
MALVELKVPDIGGHENVDIIAVEVNVGDTIAVDDTLITLETDKATMDVPAEVAGVIKEVKVKVGDKISEGGLIVVVEAEGAAAAPKAEAAAAPAQEAPKAAAPAPQAAQFGGAADAEYDVVVLGGGPGGYSAAFAAADEGLKVAIVERYKTLGGVCLNVGCIPSKALLHNAAVIDEVRHLAANGIKYPKPELDIDMLRAYKDGVVSRLTGGLAGMAKSRKVDVIQGDGQFLDPHHLEVSLTAGDAYEQAAPTGEKKIVAFKNCIIAAGSRVTKLPFIPEDPRIIDSSGALALKEVPGKLLIIGGGIIGLEMGTVYSTLGSRLDVVEMMDGLMQGADRDLVKVWQKQNEYRFDNIMVNTKTVAVEPKEDGVYVTFEGANAPKEPQRYDAVLVAAGRAPNGKLISAEKAGVAVTDRGFIEVDKQMRTNVPHIYAIGDIVGQPMLAHKAVHEGHVAAENCAGHKAYFDARVIPGVAYTSPEVAWVGETELSAKASGRKITKANFPWAASGRAIANGCDNGFTKLIFDAETGRIIGGGIVGPNGGDMIGEVCLAIEMGCDAADIGKTIHPHPTLGESIGMAAEVALGVCTDLPPQKKK

SEQ ID NO: 29 - protein, 236 aa, Neisseria gonorrhoeae (strain NCCP11945)
MTKQLKLSALFVALLASGTAVAGEASVQGYTVSGQSNEIVRNNYGECWKNAYFDKASQGRVECGDAVAVPEPEPAPVAVVEQAPQYVDETISLSAKTLFGFDKDSLRAEAQDNLKVLAQRLSRTNVQSVRVEGHTDFMGSEKYNQALSERRAYVVANNLVSNGVPASRISAVGLGESQAQMTQVCQAEVAKLGAKASKAKKREALIACIEPDRRVDVKIRSIVTRQVVPARNHHQH

SEQ ID NO: 30 - protein, 642 aa, Neisseria gonorrhoeae (strain ATCC 700825 / FA 1090)
MAKVIGIDLGTTNSCLAISENGQTKVIENAEGARTTPSIIAYLDGGEILVGAPAKRQAVTNAKNTIYAAKRLIGHKFEDKEVQRDIESMPFEIIKADNGDAWVKAQGKELSPPQISAEVLRKMKEAAEAYLGEKVTEAVITVPAYFNDSQRQATKDAGRIAGLDVKRIINEPTAAALAFGMDKGDNKDRKIAVYDLGGGTFDISIIEIANLDGDKQFEVLATNGDTFLGGEDFDQRLIDYIIDEFKKEQGIDLKQDVMALQRLKEAAEKAKIELSSGQQTEINLPYITMDATGPKHLAMKITRAKFESLVEDLIARSIEPCRTALKDAGLSTGDIDDVILVGGQSRMPKVQEAVKDFFGKEPRKDVNPDEAVAVGAAIQGEVLSGGRSDVLLLDVTPLSLGIETMGGVMTKLIQKNTTIPTKASQVFSTAEDNQSAVTIHVLQGERERASANKSLGQFNLGDIAPAPRGMPQIEVTFDIDANGILHVSAKDKGTGKAANITIQGSSGLSEEEIERMVKDAEANAEEDKKLTELVASRNQAEALIHSVKKSLADYGDKLDAAEKEKIEAALKEAEEAVKGDDKTAIDAKAEALGTASQKLGEMVYAQAQAEAQAGEGAQANASAKKDDDVVDADFEEVKDDKK

SEQ ID NO: 31 - protein, 544 aa, Neisseria gonorrhoeae
MAAKDVQFGNEVRQKMVNGVNILANAVRVTLGPKGRNVVVDRAFGGPHITKDGVTVAKEIELKDKFENMGAQMVKEVASKTNDVAGDGTTTATVLAQSIVAEGIKAVTAGMNPTDLKRGIDKAVAALVEELKNIAKPCDTSKEIAQVGSISANSDEQVGAIIAEAMEKVGKEGVITVEDGKSLENELDVVEGMQFDRGYLSPYFINDAEKQIAGLDNPFVLLFDKKISNIRDLLPVLEQVAKASRPLLIIAEDVEGEALATLVVNNIRGVLKTVAVKAPGFGDRRKAMLQDIAILTGAVVISEEVGLSLEKATLDDLGQAKRIEIGKENTTVIDGFGDAAQIEARVAEIRQQIETATSDYDKEKLQERVAKLAGGVAVIKVGAATEVEMKEKKDRVEDALHATRAAVEEGVVAGGGVALLRARAALENLHTGNADQDAGVQIVLRAVESPLRQIVANAGGEPSVVVNKVLEGKGNYGYNAGSGEYGDMIGMGVLDPAKVTRSALQHAASIAGLMLTTDCMIAEIPEEKPAVPDMGGMGGMGGMM

SEQ ID NO: 32 - protein, 96 aa, Neisseria gonorrhoeae (strain ATCC 700825 / FA 1090)
MTIRPLHDRVVVKRLEAEEKTASGIVLPGAAAEKPDMGEVIAVGAGKIGKDGARRPLDVKAGDKIIFGKYSGQTVKADGEELLVMREEDIFGIVEK

SEQ ID NO: 33 - protein, 89 aa, Neisseria gonorrhoeae (strain NCCP11945)
MNKSELIEAIAQEADISKAAAQKALDATTNAVTNALKQGDTVTLVGFGTFYVGERAERQGRNPKTGEPLTIAAAKTLKFRAGKALKDAL

SEQ ID NO: 34 - protein, 236 aa, Neisseria gonorrhoeae DGI2; identical to SEQ ID NO: 29

SEQ ID NO: 35 - protein, 801 aa, Neisseria gonorrhoeae (strain ATCC 700825 / FA 1090)
MARLFSLKPLVLALGFCFGTHCAADTVAAEEADGRVAEGGAQGASESAQASDLTLGSTCLFCSNESGSPERTEAAVQGSGEASVPEDYTRIVADRMEGQSKVKVRAEGSVIIERDGAVLNTDWADYDQSGDTVTVGDRFALQQDGTLIRGETLTYNLDQQTGEAHNVRMETEQGGRRLQSVSRTAEMLGEGRYKLTETQFNTCSAGDAGWYVKAASVEADRGKGIGVAKHAAFVFGGVPLFYTPWADFPLDGNRKSGLLVPSVSAGSDGVSLSVPYYFNLAPNFDATFAPGIIGERGATFDGQIRYLRPDYSGQTDLTWLPHDKKSGRNNRYQAKWQHRHDISDTLQAGVDFNQVSDSGYYRDFYGGEEIAGNVNLNRRVWLDYGGRAAGGSLNAGLSVQKYQTLANQSGYKDEPYAIMPRLSADWHKNAGRAQIGVSAQFTRFSHDGRQDGSRLVVYPGIKWDFSNSWGYVRPKLGLHATYYSLDSFGGKASRSVGRVLPVVNIDGGTTFERNTRLFGGGVVQTIEPRLFYNYIPAKSQNDLPNFDSSESSFGYGQLFRENLYYGNDRINAANSLSTAVQSRILDGATGEERFRAGIGQKFYFKDDAVMLDGSVGKNPRSRSDWVAFASGGIGGRFTLDSSIHYNQNDKRAEHYAVGAGYRPAPGKVLNARYKYGRNEKIYLQADGSYFYDKLSQLDLSAQWPLTRNLSAVVRYNYGFEAKKPIEMLAGAEYKSSCGCWGAGVYAQRYVTGENTYKNAVFFSLQLKDLSSVGRNPAGRMDVAVPGYIPAHSLSAGRNKRP

SEQ ID NO: 36 - protein, 635 aa, Neisseria gonorrhoeae (strain ATCC 700825 / FA 1090)
MPSEASRPVRTVLESKSATPMHDTRTMMIKPTALLLPALFFFPHAYAPAADLSENKAAGFALFKSKSPDTESVKLKPKFPVRIDTQDSEIKDMVEEHLPLITQQQEEVLDKEQTGFLAEEAPDNVKTMLRSKGYFSSKVSLTEKDGAYTVHITPGPRTKIANVGVAILGDILSDGNLAEYYRNALENWQQPVGSDFDQDSWENSKTSVLGAVTRKGYPLAKLGNTRAAVNPDTATADLNVVVDSGRPIAFGDFEITGTQRYPEQTVSGLARFQPGTPYDLDLLLDFQQALEQNGHYSGASVQADFDRLQGDRVPVKVSVTEVKRHKLETGIRLDSEYGLGGKIAYDYYNLFNKGYIGSVVWDMDKYETTLAAGISQPRNYRGNYWTSNVSYNRSTTQNLEKRAFSGGIWYVRDRAGIDARLGAEFLAEGRKIPGSDVDLGNSHATMLTASWKRQLLNNVLHPENGHYLDGKIGTTLGTFLSSTALIRTSARAGYFFTPENKKLGTFIIRGQAGYTVARDNADVPSGLMFRSGGASSVRGYELDSIGLAGPNGSVLPERALLVGSLEYQLPFTRTLSGAVFHDMGDAAANFKRMKLKHGSGLGVRWFSPLAPFSFDIAYGHSDKKIRWHISLGTRF

SEQ ID NO: 37 - protein, 467 aa, Neisseria gonorrhoeae
MKKIQADIVVIGGGTAGMGAFRNARLHSDNVYLIENNVFGTTCARVGCMPSKLLIAAAEARHHALHTDPFGVHLDKDSIVVNGEEVMRRVKSERDRFVGFVVTDVEEWPADKRIMGSAKFIDEHTVQIDDHIQIAAKSFVIATGSRPVILPQWQSLGDRLIINDDVFSWDTLPKRVAVFGPGVIGLELGQALHRLGVKVEIFGLGGIIGGISDPVVSDEAKAVFGEELKLHLDAKTEVKLDADGNVEVHWEQDGEKGVFVAEYMLAAVGRRPNVDNIGLENINIDKDARGVPVADPLTMQTSIPHIFIAGDASNQLPLLHEAADQGKIAGDNAGRYPNIGSGLRRSTIGVVFTSPQIGFVGLKYAQVAAQYQADEFVIGEVSFKNQGRSRVMLVNKGHMRLYAEKATGRFIGAEIVGPAAEHLAHLLAWAHQMKMTVPQMLDMPFYHPVIEEGLRTALRDADAKLKA

SEQ ID NO: 38 - protein, 297 aa, Neisseria gonorrhoeae
MIIAEDVEGEALATLVVNNIRGILKTVAVKAPGFGDRRKAMLQDIAILTGGVVISEEVGLSLEKATLDDLGQAKRIEIGKENTTVIDGFGDAAQIEARVAEIRQQIETATSDYDKEKLQERVAKLAGGVAVIKVGAATEVEMKEKKDRVEDALHATRAAVEEGVVAGGGVALLRARAALENLHTGNADQDAGVQIVLRAVESPLRQIVANAGGEPSVVVNKVLEGKGNYGYNAGSGEYGDMIGMGVLDPAKVTRSALQHAASIAGLMLTTDCMIAEIPEEKPAVPDMGGMGGMGGMM

SEQ ID NO: 39 - protein, 90 aa, Neisseria gonorrhoeae (strain ATCC 700825 / FA 1090)
MRKTFLILTVSAALLSGCAWETYQDGNGKTAVRQKYPAGTPVYYQDGSYSKNMNYNQYRPERRAVLPDQTGNNADEEHRQHWQKPKFQNR

SEQ ID NO: 40 - protein, 288 aa, Neisseria gonorrhoeae (strain ATCC 700825 / FA 1090)
MKTFFKTLSAAALALILAACGGQKDSAPAASAAAPSADNGAAKKEIVFGTTVGDFGDMVKEQIQAELEKKGYTVKLVEFTDYVRPNLALAEGELDINVFQHKPYLDDFKKEHNLDITEAFQVPTAPLGLYPGKLKSLEEVKDGSTVSAPNDPSNFARALVMLNELGWIKLKDGINPLTASKADIAENLKNIKIVELEAAQLPRSRADVDFAVVNGNYAISSGMKLTEALFQEPSFAYVNWSAVKTADKDSQWLKDVTEAYNSDAFKAYAHKRFEGYKYPAAWNEGAAK

SEQ ID NO: 41 - protein, 751 aa, Trichomonas vaginalis G3
MFCSLLITSAFAIHNRTENITLKDDQTLVYSHLKNGSYLMPLYVKDIWPECENDTSITFCWYYLTRGNAWDFGYAKLPNGVQHPQKGQYCTDFDVLYRGAWTTFAKTGWWPIWSIDDSIYYRIHGSENGTNTLRNVTIRTKITQPAGPNYLLIEFIAHNHDSQPHIVNVLSYTDVMIGNKDSAPIKWYPPNTHNGFSMENEEANRTLVLIGKNGFGVNPVDYLWFGLYSEGQTYKFNKTDESPTPIGRDTAFSLGWTNRRIYPGQNLSFGVLLGIGEFNQLKFPPTITVDESKFKINYAPGEKIKIPIRVQDKLTGSYGLRVTCEFPNNESKTHNISKTEGTVNEPVEFEYDLGQNISRYPVKCYAENYDITKTDHPGPKSNDFNRVFLVNEAPRLTLTSQINDQYGRGGYVNIDGIVWDDTRVTMTYQVDDNFYYRADGDITCDKQEKLFSKQIQISPSYSYGKHTLQIWAEDEFGVKSPIVKKEFSVVQNHPPEVNITEVDDNKSGNYYNSPITFKLQVRDVDVDDVILLMVKTPGTNQFAQIMTTPAKQQEWINFTYTYDVEALHEEGNYAIIFQATDRIGSPSRNKEYTFIFKKHPVPTPAQPRSEKTDNSGNIEQCAMVTDANGDSFLNCTMTHVIIDVNQKTPSASNDDGDAFSNQGDANKSNSKKKDKYLIIGIAAAAVVAAAAIIAAILIAKEASKKANDFGFNPETEEALQANNDFVQEKENPVYNENAQDDPFANEFEDVD

SEQ ID NO: 42 - protein, 748 aa, Trichomonas vaginalis G3
MLPLFYTLISSDDYIVKTKYLRAYYCRHYYYDPWTDINIQYNERADSTSGGERWVPTTYSDGGWFPIFKVDDDPTKVRILGSNRGVSNYKGIYASTNVTYHPEIGEKYLLITYSFKNQDTRPHTLHVASHTDVQIRSNDRATCKWYYGKRGLTMKDPGTGITLTLLIKGGYHVTDVDTFWFGRWQGPNTNLHYFDNYTDSGDNDLVNTDSAFSIGWLNRHIYPNETLDFSVLLGVGANLKNPAVLTVNDNFADNNMPNQEITVTGTVNDFDPDENVTVYYQFNGGPETKVETFPTGASGGISNGAFSFKVTLGPDVAQYPLKVYARDSFGLTSNVFEKNLLVNEIPRLVLTRAPPSTFFTGGTVILEGTIWDDRKATLKYQVDNGYNWNTGDEEFVCNRATKPFRKSFPIQEDYINYGHHVIKIWAQDDFGVQSEPIIAEFDYVQLHAPEMKPSQAQTSIPEVHVGKKFTISGQARDIDSGERVSVYYKYPEDTPGTQPRPLFTFDSNTGWQEWEIEYEVPDRKLPFDQEVKVILYAEDTRGGTSADLEFKFIVKKVQTIPPTPYDGEVPPNPSDNPNIPDSSYSGLTATSEVPTIVCEEHTDVNGDTYTRCDLGTTYIVITTDATPAPTQSATPSASPEPGAFPEEDNAKEVSASKEKSNKKKMLIIGLAAGGVAAAAVVAAAIIIHEATKAPKDFVFNEENGEFMEVDGDACQDADNPIYDENGADDPFANEFDEDDGPVEGIFPA

SEQ ID NO: 43 - protein, 613 aa, Trichomonas vaginalis G3
MFNLFLATVSSEKRPQIEADKVRFQGYGKFSKTGHQIAISSNQRLYYYASVHIINAYFSNCVANDLNLKWQMSCGGAIFLNKGSLYFERKDGSYSSSFDQCQATDKGGAIYAYDSACDIFQVNFFRCKAGNEGGAYYHDGMRYSRPYYANAKYNTLIIEYCTFKGNLADSYGGALAVKGAVPFTLKNSKFLNNGAVAGGALYGDYSDITMTNNLFVLNFGDHTRPCQNNKKCGSPNYQSFKYVPAGAILIRSSPEYFPVDVYSAENCFNQNFLLNNRWPDKSKTSVNILLLFAVRFKSVNDKMKWHTVNVIDNMTLAKKFNYPKEYPSKYIQLRANGINIRSFEMTGTRQDVEGCKIDGFPAVTPIPPATPIPTPYPTVPTPDPTQPPPPTRSLAATPYPTIPPPRTPFPSATIPPATKKKDTPFPTLAPPQTPAPTPSPIPTREPTAPPTATPAATRSAIPTPISVPPTINITIPANASVDEEINTSDCGEMCKTEHIPMRTPNAITINYESPVPNTEDSANNAKNAVIGRNTAAPDESAVGFVIAAVAAVAAVGVIAGIIYTLTRSKPPPMDLENAERVNMGNDNNAVENDNPIYNNNAAQDPFADEFEDA

SEQ ID NO: 44 - protein, 596 aa, Trichomonas vaginalis G3
MSSDKSSRVTSEENIEKTTTTGFEMFECLKLFRNKAILFLVYFISLGNGALPIFNMMILGDVTSSASTDPTKTATKLMTPLLLKLTYISIAQAVILLITIMCKSYIIPTFTVDIRQAMFNSIMTQPIDFFDKTSSGVLMGRFSEDITIIRDVYIEKNCAMLQGMTMSLIAIIMGFIRLPYVSLSYFVAIPLLVASYILSEKYIDKLWKNHNIQSTSIASKTEEVISQYRTVKAFDCEKKECDDYNDLLDNVDDIYRKTAIAQGLKEAFSSIIANGLTVFVVYFIAYLMMVKKNTKVKSGDSLSMMMYIMLGTMGFSQILSASDSYKKANMAALKILNIINRKVENDSENQTEIGKIEGKIEFQNVSFKYSTRDEYAIRNLTFEIKPGETVALVGESGCGKTTTLSLLQRFYDVSEGKILIDGKDISNFSASSLRSQISCVPQSPVLFSMSILDNVKYGKPESSFDEVKTAAEIGNAHNFICQMENQYDQEVQQISLSGGQKQRICISRAVLCNAPILLLDEATASLDAESEQLVQESLEKVRKGKTAIIVAHRLSTVKNADRILVFDNGTIVETGTHEELLEKGGIYSNLVKFQLQ

SEQ ID NO: 45 - protein, 846 aa, Trichomonas vaginalis G3
MYLGFLISFASSNQNKPVLENCNYYSTYNYSCATIPSGMNYIDGLLRCNSSSQVIDLTSDEMTCIDYASGTKVLYDTAVVSENTTGLSSKMIVFFDQSDKFSSRLSTDYGNLLDDAVKACKSNYAQMYTPCQIVASGCALSSYYPHSPACIAYNALPAANSTTYEYKYWPANRPFIEYGVQASKVIDEHIMNTTFSKEEQINIVLARYSQNGTFLGYVPLTNQFDICTEKRDVNLMWQLYGTGYVSECEVNIMDIFNSTTTDVYDPFLVQEVSGTNVLRPIPVNVLSYRDANEIPVNQRSIERKKRLFRRFFALDNYTNPIFIQYLSSMSIKFEHFNETSEERIPVITVGYTTVRRSDLQESDYPIYLDVESFTTSNYSFSIEFSTNIESYWEAALITLIVLAIICIIIWLYRAVVTVKRYGTEGIDFKVIAALFAEAFNIVAWLLFIMAFVFSFAIFCAYKWTPSSKYTILGNEFGILTGFIWAAWVLSFIGLVIKYVLMLTSETFLIDWEPRRPSIPVSAWRRILVGNEFLKLHTRRSYNIPFTVITLVFILGGFGVDKLQAVLPSSTLIESGSNYGVLRFAIVTFIYILLLIFQYIVTRIVWLISGSPYEDFARLCGTANVSVLTLLSPSWAIYLNGRAMKPADEGDIKLIQSISEAEKGALSIKPLSENRPEQVYECFFAPKLREPLYQAYDRIVEMHHMRPKNLKRANTSIVSLEAMSSFEQLNVFLQRFFGAEGKDREYDVWKTPFGYKLSRMPPEPPERSLLYAQSTNSLRKAIDGYGEWLLALFDLLLFVCVDYQASSTPIAAFVTLIIDAVMMAAWRSAAKRNLARKSLIDNRFFLN

SEQ ID NO: 46 - protein, 454 aa, Trichomonas vaginalis G3
MGEDVSEVDEQSPKSNLLKWIFIAVAVVVVIVIIVTVTVVLVLKKKRNEKYPGFLYLNDIHIDLSYNPKSNKDWCHSQTNNLLESWEFGQYNCDPPPKLYDSLVESLKTNVPSVDFILLGGDLPSHDLGGNYTFLKEHFRLITDPLEKLYPNKKIFITLGNNDFQENYGSFKTDLKDFENAHEVFGKWMNEEQSKTFKKGGYYYEDMPELKLRLLLLNTVMYTNTKSRVFNESLKDPYDQFAWIRQTYKEGVDKGYKVGVALHVPPGIVYYKGIPGFPSMYLEEFGKVFEECDFSFTISGHSHIDTLNPLYKANVEEDNIQYSLSAVSVSPSHYNNPGYRYFEIKDGVLQDYTQFYADIMMNPDSPKWEVEYKFRDAYKVKDLSKKSLNDATRYIRSKGSVIWSYRGYIYSQAEKYNPFFYCALRALTKEDVFKCSLDLNVNLSSIMPYSNRGD

SEQ ID NO: 47 - protein, 1576 aa, Trichomonas vaginalis G3
MNPSESSVSKSTSSVSSIGVNKDSVIQGKYSLSDQIFPVYDQMMQKAILPKWFLAFVAFYIMLQILIIAFWVYTEPFLRINSKYSKFFEIFLKVFIYGDAIHYTEVKGLNMYRTLIVSLFAFFWVFFVIYYHKLKYSIPVPLLYITSLIVDILVPVFITPSAYVACHGIVNLKYAHNSTIIGEIIIGFISYGITLMNFSITTTLKARSVALTNLTFPLFDSSSIVVWTISTTLCCILSAILTYFENWTQIIVIVIHAIISCYLCYRLLFIPFYDLYRNASVLAFAITSIVLDIYSILMQLIKSIPYEYIPFILIGSLIISFIFASIFYKRKVKQIKEDLTFRTDNPKAPEYLASLNIDSTQLRAMEYIVVGLTQICDYFVDGSLTDYIIKVDEFEGILAILLQVVTFFPCESRKMDVLYKKLIMKRKLSFADRFLLYQVYRIKTRRLVTDTKSTLETYTKLKARNDECKQSIRSFWDFPSCKINYLSSLSITVNDINSLFINTIQENPNNVRIATEYSDFLIECMTNFDEAIRQKVKVERILNGTNFNVDISFRSLVNKFPRYLKDKILDTKGRLIMRLKERNSDPLNDNSSNQSKSGSSSKETNTSTLTVDLETQEVVSKRVLRDSKVRLAFHQSIHTLHPHHMKNLTILANSILVVCFSIFIAYYAYQKDKLKWRRDAFVEFRYMSLALDKTYYASFVLTLEWARMHDRYDNSTEIMGNISIDFEDNPIAKNKWEPAYETIYQTVDQAKDFLETLYQSMADSARTEDIYEIIPLLLKPRSKIYACTNYEISHDMPGNLKDQFVIIHFFQDNFAGDFHVMDKDIPNIYQNDFYCQLFANSYILSKNAEESIENILDYSVEKSQKLIDDVWLWTGIGGGIVLFVTFIPMIIIIINYYKIVNGLLKVLLELPNSAKEDAKKRLNIENTDEIVETSNKTKKSKLLEISIFIYFASAALITVLYCLSGLYTYYFNDLMANLLDWYYISCVRNVASSELRNNILHIILLNDSLPNKIIPLEDIYQAALDEIDLLKRYNQYLIEGGNNFERFIGFDAESDSYQFMEVCELGRDPKSMHDMYACSSIDKQIAFLTTNVRDIMKNPDKLSGAINDEVTQNVMHLINNHFYPLTVLAATRVKSLLQDNFDAGMKKLTIYLVIELLISLFLFILPLFIRAVIWENYKMLLMLLKHLPPQVIIDTPEILDFFREKSKHHHTEAMTISKSVVYNTSECIAITNQNAIIEIVNQSLTANINITPDQILGQSITNIISLSEHDRIGNQIQLMTTGQGSSVWQDHTKLVKDDGSEVPFGITIIGMKENEGSADITSLVFILENEEEKIKQKKLAEESKAKSEKLLYQILPKDIVVRLNRGETDISFTIPSATIFFIDIVKFSSYAELLTPSEIMANLSLVFATFDGIVSEFQSITKIKLIGDVYMAAAGLFQDPKEESKQHAEDAVRCCLKCAKSMEEINMKLNASLEVRIGCNSGGPLIGGVLGTDKPTFDIIGDTINVAARLQSTDIPGNVQISASTKEMIEHLDFVIEERGLIYLKGKGKQMTYFVSFKNNDGNKSSFDSSFTLKLN

SEQ ID NO: 48 - protein, 370 aa, Trichomonas vaginalis G3
MFRQLLAGSLPTDMIVPNFTHVYPECDKKLEKTMNFTTLYTKELEAGEIICFYKTYAIAGNAAYTVNATYFNPENTSIYETKFAESPFLVSGPISPKVIPVSKVACKDSSKKCKIQFISITPSGHQKLEESDLYVDNIFDSYLSTKKKQSFSKSYSMEFHISSKNNKVKRVMNSSTFISTHIGSKSRTITVSPDSLYVFADGKKQEKNTGTGKALSFAPSQEFSLSLVNMSELQTKIQTDKKDGKINDSYKIDKKGSQTITVSISEPKSSSEDEEFFFDEDKEYYLKGDASLKSKKEVEEDTKENPPPGSSFPAWEIAVIVIVIILIIVIIIIIIFCCCCCCCSCCSCKKGSSNVGSAKDDEDSGSGVNV

SEQ ID NO: 49 - protein, 567 aa, Trichomonas vaginalis
MLASSVAAPVRNICRAKLPALKTGMTLLQDGDLSKGSAFTKEERDRLNLRGLLPYKVFTKDEQAARIRRQFELMPTPLLKYIFLANEREKNSQSFWRFLFTHPPTETMPVLYTPTVGEACQKWATHRQSYRGIYITPEDSGKIKDILRNYPRQDIRCIVVTDGGRILGLGDLGASGLGIPVGKLMLYTLIGQVHPDQTLPVQLDMGTDRKEILADPLYHGWRHPRIRGPEHTKFVAEFVDAVKEVFGETCLVQFEDFEMETAFKLLDHFRWRCNCFNDDIEGTAAVAAATLASATHMEGVPDLKNQKIIFIGAGSAATGIANLIVDMAVSRGGISRKDAERNIIMFDHKGMVHADRKDLYDFNKPYMHDMEVYGSVLEGVKKFKATCVIGVSGVPGLITKEIVQATCANCERPVIMPLSNPTVKAEAKPHDVYQWSNGKALCATGSPFPVETVNGKKTITAQANNSWIFPAVGYALVTTRARHCPGKVFEVAAESLASLVKKEDHDMGNLLPPLDKIREYSFGIALDVAKYLIKNELATALPPKGTELKDWLKAQLFDPQAEYEQLY

SEQ ID NO: 50 - protein, 309 aa, Trichomonas vaginalis
MLSSSFERNLHQPLLFIDKDTKVVIQGIGNQGQFHSRLMRQYGTKVVGAVHPKKAGSIIAGLPIFKNMKEVVKRTDANASLIFVPAPGAAAACIEAAQAGMGLVVCITEHIPQHDMIKVKKVMKETGCQLIGPNCPGLIQPGTHTKLGIIPTNIFNNGKIGIVSRSGTLTYEAAYATTLAGLGQSTVVGIGGDPFAGQLHTDVVKRFAADPQTEGIILIGEIGGTSEEDAAEWIAKTKLTQEKPVVAFIAGATAPPGKRMGHSGAIVSGGKGTAEGKYKALEAAGVRIARHPGNMGKFIFEEMKRMGKI

SEQ ID NO: 51 - protein, 931 aa, Trichomonas vaginalis
MSVRREGLLDDAWEKTQIKVFSRWVQKQLLARQIQFETIETDFEDGTKLLNLLEIIGKEPMPSKWHKQPKMMVQKRENVDLALKYINEVKKIRTVGIGADDIINKNLKLTLGLTWTCINKFMIEEISVEEATARDALLLWAKKNTQGYEHVAVNNFTTSWNTGLAFAALINKFRPNLLDYSALDYNDHKGACEKAFAACKELGIYVYLDPEDVIDTTPDEKSVVTQVAEFFHFFASESKIAAMADKIKRTVAIQKQIDELKNTYIEDAKAAIEKMTVEDEKLKADDYEKTIPGIRGKLASVISYNRDIRPEIVDHRAKAMRSWAALVTKCKSGNRPIPEIPQGLEPEALTNKFNEIEQTSTTRRDELTQELNDMIKKKVEDFMAKCMDIINKCDAIHEEVKTIEGTTAEKKDKVEQKLHEAEDLQPALAELTPLFQELVELRINTLSSQTDDSVNRHHSQLITYIKHLLEQLNGKLFEETNEARINEYNALAQPLYDEAIAFKEEVLAISGELRERRTQFLAKQAEAPTKREHVNEIDPIFDGLEKDSLHLRVNHSPTEIRNVYAVTLQHIITELNKIFEEMVANFDATAVPIIDGITALVTSSHQIPGDAAAVKAQVEENLASLDGFAEKIQALQDPYNELVEFKLNYKVTYTYSDATGELDQARLDLKQIILAKKTFLEEEERKARINNYTVKADEHMNEAHALDGKINSVDGELEPKRQKLYEVREEVNAKKEKAAEELTPIYEDLEKDQLHLEITSTPASINIFFENLIAHIDTLVKEIDAAIAAAKGLEISEEELNEFKDTFKYFDKDKSNSLEYFELKACLTALGEDITDGQAKEYCKKYNSKGEGTALEFDDYVRFMLDHFSKAETTETTMEAFKAIAQNQPVLTDAQLDQYFSAEDAAYLRSQLKQGENGYEFADWVNSLYNH

SEQ ID NO: 52 - protein, 792 aa, Neisseria gonorrhoeae; identical to SEQ ID NO: 23

SEQ ID NO: 53 - protein, 792 aa, Neisseria gonorrhoeae; identical to SEQ ID NO: 24

SEQ ID NO: 54 - protein, 326 aa, Neisseria gonorrhoeae; identical to SEQ ID NO: 25

SEQ ID NO: 55 - protein, 392 aa, Neisseria gonorrhoeae; identical to SEQ ID NO: 26

SEQ ID NO: 56 - protein, 467 aa, Neisseria gonorrhoeae; identical to SEQ ID NO: 27

SEQ ID NO: 57 - protein, 594 aa, Neisseria gonorrhoeae (strain ATCC 700825 / FA 1090); identical to SEQ ID NO: 28

SEQ ID NO: 58 - protein, 236 aa, Neisseria gonorrhoeae (strain NCCP11945); identical to SEQ ID NO: 29

SEQ ID NO: 59 - protein, 642 aa, Neisseria gonorrhoeae (strain ATCC 700825 / FA 1090); identical to SEQ ID NO: 30

SEQ ID NO: 60 - protein, 544 aa, Neisseria gonorrhoeae; identical to SEQ ID NO: 31

SEQ ID NO: 61 - protein, 96 aa, Neisseria gonorrhoeae (strain ATCC 700825 / FA 1090); identical to SEQ ID NO: 32

SEQ ID NO: 62 - protein, 89 aa, Neisseria gonorrhoeae (strain NCCP11945); identical to SEQ ID NO: 33

SEQ ID NO: 63 - protein, 236 aa, Neisseria gonorrhoeae (strain ATCC 700825 / FA 1090); identical to SEQ ID NO: 29

SEQ ID NO: 64 - protein, 801 aa, Neisseria gonorrhoeae (strain ATCC 700825 / FA 1090); identical to SEQ ID NO: 35

SEQ ID NO: 65 - protein, 88 aa, Chlamydia trachomatis; identical to SEQ ID NO: 3

SEQ ID NO: 66 - protein, 512 aa, Chlamydia trachomatis (strain D/UW-3/Cx); identical to SEQ ID NO: 4

SEQ ID NO: 67 - protein, 394 aa, Chlamydia trachomatis serovar L2 (strain 434/Bu/ATCC VR-902-B); identical to SEQ ID NO: 5

SEQ ID NO: 68 - protein, 102 aa, Chlamydia trachomatis (strain D/UW-3/Cx); identical to SEQ ID NO: 6

SEQ ID NO: 69 - protein, 102 aa, Chlamydia trachomatis; identical to SEQ ID NO: 6

SEQ ID NO: 70 - protein, 89 aa, Chlamydia trachomatis; identical to SEQ ID NO: 8

SEQ ID NO: 71 - protein, 660 aa, Chlamydia trachomatis serovar L2 (strain 434/Bu/ATCC VR-902-B); identical to SEQ ID NO: 19

SEQ ID NO: 72 - protein, 232 aa, Chlamydia trachomatis serovar L2 (strain 434/Bu/ATCC VR-902-B); identical to SEQ ID NO: 20

SEQ ID NO: 73 - protein, 1014 aa, Chlamydia trachomatis serovar A (strain A2497); identical to SEQ ID NO: 21

SEQ ID NO: 74 - protein, 547 aa, Chlamydia trachomatis; identical to SEQ ID NO: 22

SEQ ID NO: 75 - protein, 635 aa, Neisseria gonorrhoeae (strain ATCC 700825 / FA 1090); identical to SEQ ID NO: 36

SEQ ID NO: 76 - protein, 467 aa, Neisseria gonorrhoeae; identical to SEQ ID NO: 37

SEQ ID NO: 77 - protein, 297 aa, Neisseria gonorrhoeae; identical to SEQ ID NO: 38

SEQ ID NO: 78 - protein, 90 aa, Neisseria gonorrhoeae (strain ATCC 700825 / FA 1090); identical to SEQ ID NO: 39

SEQ ID NO: 79 - protein, 288 aa, Neisseria gonorrhoeae (strain ATCC 700825 / FA 1090); identical to SEQ ID NO: 40

SEQ ID NO: 80 - protein, 751 aa, Trichomonas vaginalis G3; identical to SEQ ID NO: 41

SEQ ID NO: 81 - protein, 748 aa, Trichomonas vaginalis G3; identical to SEQ ID NO: 42

SEQ ID NO: 82 - protein, 613 aa, Trichomonas vaginalis G3; identical to SEQ ID NO: 43

SEQ ID NO: 83 - protein, 596 aa, Trichomonas vaginalis G3; identical to SEQ ID NO: 44

SEQ ID NO: 84 - protein, 846 aa, Trichomonas vaginalis G3; identical to SEQ ID NO: 45

SEQ ID NO: 85 - protein, 454 aa, Trichomonas vaginalis G3; identical to SEQ ID NO: 46

SEQ ID NO: 86 - protein, 1576 aa, Trichomonas vaginalis G3; identical to SEQ ID NO: 47

SEQ ID NO: 87 - protein, 370 aa, Trichomonas vaginalis G3; identical to SEQ ID NO: 48

SEQ ID NO: 88 - protein, 567 aa, Trichomonas vaginalis; identical to SEQ ID NO: 49

SEQ ID NO: 89 - protein, 309 aa, Trichomonas vaginalis; identical to SEQ ID NO: 50

SEQ ID NO: 90 - protein, 931 aa, Trichomonas vaginalis; identical to SEQ ID NO: 51